European Patent Application EP 4 368 628 A1, published May 15, 2024. Title: Methods and apparatus for purification of nucleotides, hydrophobic reagents and hydrophobic substrates. Applicant: JAPAN SCIENCE AND TECHNOLOGY AGENCY. The sequence listing filed with the application follows.

SEQUENCE LISTING (19 sequences)

SEQ ID NO: 1 - DNA, 18 bp, synthetic construct
  misc_feature 1..18: note = T7 Promoter
  source 1..18: mol_type = other DNA
taatacgactcactatag

SEQ ID NO: 2 - DNA, 19 bp, synthetic construct
  misc_feature 1..19: note = artificial sequence
  misc_feature 1: note = Phosphate protector bound to the 5' end
  source 1..19: mol_type = other DNA
taatacgactcactatagg

SEQ ID NO: 3 - DNA, 20 bp, synthetic construct
  misc_feature 1..20: note = KOD-Plus-Neo (TOYOBO), Fw primer
  source 1..20: mol_type = other DNA
cgcgcgttggccgattcatt

SEQ ID NO: 4 - DNA, 100 bp, synthetic construct
  misc_feature 1..100: note = KOD-Plus-Neo (TOYOBO), Rev primer
  source 1..100: mol_type = other DNA
ttttttttttttttttttttttttttttttttttttttttttttttttttttttttttttttttttttttttttttttttcagttagacgttgatcctgg

SEQ ID NO: 5 - DNA, 4411 bp, synthetic construct
  misc_feature 1..4411: note = pSP73-a-luc2
  source 1..4411: mol_type = other DNA
tatagtgtcacctaaatcgtatgtgtatgatacataaggttatgtattaattgtagccgcgttctaacgacaatatgtccatatggtgcactctcagtacaatctgctctgatgccgcatagttaagccagccccgacacccgccaacacccgctgacgcgccctgacgggcttgtctgctcccggcatccgcttacagacaagctgtgaccgtctccgggagctgcatgtgtcagaggttttcaccgtcatcaccgaaacgcgcgagacgaaagggcctcgtgatacgcctatttttataggttaatgtcatgataataatggtttcttagacgtcaggtggcacttttcggggaaatgtgcgcggaacccctatttgtttatttttctaaatacattcaaatatgtatccgctcatgagacaataaccctgataaatgcttcaataatattgaaaaaggaagagtatgagtattcaacatttccgtgtcgcccttattcccttttttgcggcattttgccttcctgtttttgctcacccagaaacgctggtgaaagtaaaagatgctgaagatcagttgggtgcacgagtgggttacatcgaactggatctcaacagcggtaagatccttgagagttttcgccccgaagaacgttttccaatgatgagcacttttaaagttctgctatgtggcgcggtattatcccgtattgacgccgggcaagagcaactcggtcgccgcatacactattctcagaatgacttggttgagtactcaccagtcacagaaaagcatcttacggatggcatgacagtaagagaattatgcagtgctgccataaccatgagtgataacactgcggccaacttacttctgacaacgatcggaggaccgaaggagctaaccgcttttttgcacaacatgggggatcatgtaactcgccttgatcgttgggaaccggagctgaatgaagccataccaaacgacgagcgtgacaccacgatgcctgtagcaatggcaacaacgttgcgcaaactattaactggcgaactacttactctagcttcccggcaacaattaatagactggatggaggcggataaagttgcaggaccacttctgcgctcggcccttccggctggctggtttattgctgataaatctggagccggtgagcgtgggtctcgcggtatcattgcagcactggggccagatggtaagccctcccgtatcgtagttatctacacgacggggagtcaggcaactatggatgaacgaaatagacagatcgctgagataggtgcctcactgattaagcattggtaactgtcagaccaagtttactcatatatactttagattgatttaaaacttcatttttaatttaaaaggatctaggtgaagatcctttttgataatctcatgaccaaaatcccttaacgtgagttttcgttccactgagcgtcagaccccgtagaaaagatcaaaggatcttcttgagatcctttttttctgcgcgtaatctgctgcttgcaaacaaaaaaaccaccgctaccagcggtggtttgtttgccggatcaagagctaccaactctttttccgaaggtaactggcttcagcagagcgcagataccaaatactgttcttctagtgtagccgtagttaggccaccacttcaagaactctgtagcaccgcctacatacctcgctctgctaatcctgttaccagtggctgctgccagtggcgataagtcgtgtcttaccgggttggactcaagacgatagttaccggataaggcgcagcggtcgggctgaacggggggttcgtgcacacagcccagcttggagcgaacgacctacaccgaactgagatacctacagcgtgagctatgagaaagcgccacgcttcccgaagggagaaaggcggacaggtatccggtaagcggcagggtcggaacaggagagcgcacgagggagcttccagggggaaacgcctggtatctttatagtcctgtcgggtttcgccacctctgacttgagcgtcgatttttgtgatgctcgtcaggggggcggagcctatggaaaaacgccagcaacgcggcctttttacggttcctggccttttgctggccttttgctcacatgttctttcctgcgttatcccctgattctgtggataaccgtattaccgcctttgagtgagctgataccgctcgccgcagccgaacgaccgagcgcagcgagtcagtgagcgaggaagcggaagagcgcccaatacgcaaaccgcctctccccgcgcgttggccgattcattaatgcaggttaacctggcttatcgaaattaatacgactcactatagggggacatcgtagagagtcgtacttagagaataaactagtattcttctggtccccacagactcagagagaacccgccaccatggaagatgccaaaaacattaagaagggcccagcgccattctacccactcgaagacgggaccgccggcgagcagctgcacaaagccatgaagcgctacgccctggtgcccggcaccatcgcctttaccgacgcacatatcgaggtggacattacctacgccgagtacttcgagatgagcgttcggctggcagaagctatgaagcgctatgggctgaatacaaaccatcggatcgtggtgtgcagcgagaatagcttgcagttcttcatgcccgtgttgggtgccctgttcatcggtgtggctgtggccccagctaacgacatctacaacgagcgcgagctgctgaacagcatgggcatcagccagcccaccgtcgtattcgtgagcaagaaagggctgcaaaagatcctcaacgtgcaaaagaagctaccgatcatacaaaagatcatcatcatggatagcaagaccgactaccagggcttccaaagcatgtacaccttcgtgacttcccatttgccacccggcttcaacgagtacgacttcgtgcccgagagcttcgaccgggacaaaaccatcgccctgatcatgaacagtagtggcagtaccggattgcccaagggcgtagccctaccgcaccgcaccgcttgtgtccgattcagtcatgcccgcgaccccatcttcggcaaccagatcatccccgacaccgctatcctcagcgtggtgccatttcaccacggcttcggcatgttcaccacgctgggctacttgatctgcggctttcgggtcgtgctcatgtaccgcttcgaggaggagctattcttgcgcagcttgcaagactataagattcaatctgccctgctggtgcccacactatttagcttcttcgctaagagcactctcatcgacaagtacgacctaagcaacttgcacgagatcgccagcggcggggcgccgctcagcaaggaggtaggtgaggccgtggccaaacgcttccacctaccaggcatccgccagggctacggcctgacagaaacaaccagcgccattctgatcacccccgaaggggacgacaagcctggcgcagtaggcaaggtggtgcccttcttcgaggctaaggtggtggacttggacaccggtaagacactgggtgtgaaccagcgcggcgagctgtgcgtccgtggccccatgatcatgagcggctacgttaacaaccccgaggctacaaacgctctcatcgacaaggacggctggctgcacagcggcgacatcgcctactgggacgaggacgagcacttcttcatcgtggaccggctgaagagcctgatcaaatacaagggctaccaggtagccccagccgaactggagagcatcctgctgcaacaccccaacatcttcgacgccggggtcgccggcctgcccgacgacgatgccggcgagctgcccgccgcagtcgtcgtgctggaacacggtaaaaccatgaccgagaaggagatcgtggactatgtggccagccaggttacaaccgccaagaagctgcgcggtggtgttgtgttcgtggacgaggtgcctaaaggactgaccggcaagttggacgcccgcaagatccgcgagattctcattaaggccaagaagggcggcaagatcgccgtgtaataattctagactggtactgcatgcacgcaatgctagctgcccctttcccgtcctgggtaccccgagtctcccccgacctcgggtcccaggtatgctcccacctccacctgccccactcaccacctctgctagttccagacacctcccaagcacgcagcaatgcagctcaaaacgcttagcctagccacacccccacgggaaacagcagtgattaacctttagcaataaacgaaagtttaactaagctatactaaccccagggttggtcaatttcgtgccagccacaccctggagaattcgagacgagatctggttc

SEQ ID NO: 6 - protein, 550 aa, synthetic construct
  REGION 1..550: note = Luc2
MEDAKNIKKGPAPFYPLEDGTAGEQLHKAMKRYALVPGTIAFTDAHIEVDITYAEYFEMSVRLAEAMKRYGLNTNHRIVVCSENSLQFFMPVLGALFIGVAVAPANDIYNERELLNSMGISQPTVVFVSKKGLQKILNVQKKLPIIQKIIIMDSKTDYQGFQSMYTFVTSHLPPGFNEYDFVPESFDRDKTIALIMNSSGSTGLPKGVALPHRTACVRFSHARDPIFGNQIIPDTAILSVVPFHHGFGMFTTLGYLICGFRVVLMYRFEEELFLRSLQDYKIQSALLVPTLFSFFAKSTLIDKYDLSNLHEIASGGAPLSKEVGEAVAKRFHLPGIRQGYGLTETTSAILITPEGDDKPGAVGKVVPFFEAKVVDLDTGKTLGVNQRGELCVRGPMIMSGYVNNPEATNALIDKDGWLHSGDIAYWDEDEHFFIVDRLKSLIKYKGYQVAPAELESILLQHPNIFDAGVAGLPDDDAGELPAAVVVLEHGKTMTEKEIVDYVASQVTTAKKLRGGVVFVDEVPKGLTGKLDARKIREILIKAKKGGKIAV

SEQ ID NO: 7 - DNA, 2167 bp, synthetic construct
  misc_feature 1..2167: note = Luc2 mRNA templete DNA
  source 1..2167: mol_type = other DNA
cgcgcgttggccgattcattaatgcaggttaacctggcttatcgaaattaatacgactcactatagggggacatcgtagagagtcgtacttagagaataaactagtattcttctggtccccacagactcagagagaacccgccaccatggaagatgccaaaaacattaagaagggcccagcgccattctacccactcgaagacgggaccgccggcgagcagctgcacaaagccatgaagcgctacgccctggtgcccggcaccatcgcctttaccgacgcacatatcgaggtggacattacctacgccgagtacttcgagatgagcgttcggctggcagaagctatgaagcgctatgggctgaatacaaaccatcggatcgtggtgtgcagcgagaatagcttgcagttcttcatgcccgtgttgggtgccctgttcatcggtgtggctgtggccccagctaacgacatctacaacgagcgcgagctgctgaacagcatgggcatcagccagcccaccgtcgtattcgtgagcaagaaagggctgcaaaagatcctcaacgtgcaaaagaagctaccgatcatacaaaagatcatcatcatggatagcaagaccgactaccagggcttccaaagcatgtacaccttcgtgacttcccatttgccacccggcttcaacgagtacgacttcgtgcccgagagcttcgaccgggacaaaaccatcgccctgatcatgaacagtagtggcagtaccggattgcccaagggcgtagccctaccgcaccgcaccgcttgtgtccgattcagtcatgcccgcgaccccatcttcggcaaccagatcatccccgacaccgctatcctcagcgtggtgccatttcaccacggcttcggcatgttcaccacgctgggctacttgatctgcggctttcgggtcgtgctcatgtaccgcttcgaggaggagctattcttgcgcagcttgcaagactataagattcaatctgccctgctggtgcccacactatttagcttcttcgctaagagcactctcatcgacaagtacgacctaagcaacttgcacgagatcgccagcggcggggcgccgctcagcaaggaggtaggtgaggccgtggccaaacgcttccacctaccaggcatccgccagggctacggcctgacagaaacaaccagcgccattctgatcacccccgaaggggacgacaagcctggcgcagtaggcaaggtggtgcccttcttcgaggctaaggtggtggacttggacaccggtaagacactgggtgtgaaccagcgcggcgagctgtgcgtccgtggccccatgatcatgagcggctacgttaacaaccccgaggctacaaacgctctcatcgacaaggacggctggctgcacagcggcgacatcgcctactgggacgaggacgagcacttcttcatcgtggaccggctgaagagcctgatcaaatacaagggctaccaggtagccccagccgaactggagagcatcctgctgcaacaccccaacatcttcgacgccggggtcgccggcctgcccgacgacgatgccggcgagctgcccgccgcagtcgtcgtgctggaacacggtaaaaccatgaccgagaaggagatcgtggactatgtggccagccaggttacaaccgccaagaagctgcgcggtggtgttgtgttcgtggacgaggtgcctaaaggactgaccggcaagttggacgcccgcaagatccgcgagattctcattaaggccaagaagggcggcaagatcgccgtgtaataattctagactggtactgcatgcacgcaatgctagctgcccctttcccgtcctgggtaccccgagtctcccccgacctcgggtcccaggtatgctcccacctccacctgccccactcaccacctctgctagttccagacacctcccaagcacgcagcaatgcagctcaaaacgcttagcctagccacacccccacgggaaacagcagtgattaacctttagcaataaacgaaagtttaactaagctatactaaccccagggttggtcaatttcgtgccagccacaccaaaaaaaaaaaaaaaaaaaaaaaaaaaaaaaaaaaaaaaaaaaaaaaaaaaaaaaaaaaaaaaaaaaaaaaaaaaaaaaa

SEQ ID NO: 8 - RNA, 2102 nt, synthetic construct
  misc_feature 1..2102: note = Luc2 mRNA
  source 1..2102: mol_type = other RNA
gggggacatcgtagagagtcgtacttagagaataaactagtattcttctggtccccacagactcagagagaacccgccaccatggaagatgccaaaaacattaagaagggcccagcgccattctacccactcgaagacgggaccgccggcgagcagctgcacaaagccatgaagcgctacgccctggtgcccggcaccatcgcctttaccgacgcacatatcgaggtggacattacctacgccgagtacttcgagatgagcgttcggctggcagaagctatgaagcgctatgggctgaatacaaaccatcggatcgtggtgtgcagcgagaatagcttgcagttcttcatgcccgtgttgggtgccctgttcatcggtgtggctgtggccccagctaacgacatctacaacgagcgcgagctgctgaacagcatgggcatcagccagcccaccgtcgtattcgtgagcaagaaagggctgcaaaagatcctcaacgtgcaaaagaagctaccgatcatacaaaagatcatcatcatggatagcaagaccgactaccagggcttccaaagcatgtacaccttcgtgacttcccatttgccacccggcttcaacgagtacgacttcgtgcccgagagcttcgaccgggacaaaaccatcgccctgatcatgaacagtagtggcagtaccggattgcccaagggcgtagccctaccgcaccgcaccgcttgtgtccgattcagtcatgcccgcgaccccatcttcggcaaccagatcatccccgacaccgctatcctcagcgtggtgccatttcaccacggcttcggcatgttcaccacgctgggctacttgatctgcggctttcgggtcgtgctcatgtaccgcttcgaggaggagctattcttgcgcagcttgcaagactataagattcaatctgccctgctggtgcccacactatttagcttcttcgctaagagcactctcatcgacaagtacgacctaagcaacttgcacgagatcgccagcggcggggcgccgctcagcaaggaggtaggtgaggccgtggccaaacgcttccacctaccaggcatccgccagggctacggcctgacagaaacaaccagcgccattctgatcacccccgaaggggacgacaagcctggcgcagtaggcaaggtggtgcccttcttcgaggctaaggtggtggacttggacaccggtaagacactgggtgtgaaccagcgcggcgagctgtgcgtccgtggccccatgatcatgagcggctacgttaacaaccccgaggctacaaacgctctcatcgacaaggacggctggctgcacagcggcgacatcgcctactgggacgaggacgagcacttcttcatcgtggaccggctgaagagcctgatcaaatacaagggctaccaggtagccccagccgaactggagagcatcctgctgcaacaccccaacatcttcgacgccggggtcgccggcctgcccgacgacgatgccggcgagctgcccgccgcagtcgtcgtgctggaacacggtaaaaccatgaccgagaaggagatcgtggactatgtggccagccaggttacaaccgccaagaagctgcgcggtggtgttgtgttcgtggacgaggtgcctaaaggactgaccggcaagttggacgcccgcaagatccgcgagattctcattaaggccaagaagggcggcaagatcgccgtgtaataattctagactggtactgcatgcacgcaatgctagctgcccctttcccgtcctgggtaccccgagtctcccccgacctcgggtcccaggtatgctcccacctccacctgccccactcaccacctctgctagttccagacacctcccaagcacgcagcaatgcagctcaaaacgcttagcctagccacacccccacgggaaacagcagtgattaacctttagcaataaacgaaagtttaactaagctatactaaccccagggttggtcaatttcgtgccagccacaccaaaaaaaaaaaaaaaaaaaaaaaaaaaaaaaaaaaaaaaaaaaaaaaaaaaaaaaaaaaaaaaaaaaaaaaaaaaaaaaa

SEQ ID NO: 9 - DNA, 676 bp, synthetic construct
  misc_feature 1..676: note = NLuc mRNA templete DNA
  source 1..676: mol_type = other DNA
cccggatcctaatacgactcactataggcgcatattaaggtgacgcgtgtggcctcgaacaccgagcgaccctgcagcgacccgcttaaaagcttggcaatccggtactgttggtaaagccaccatggtcttcacactcgaagatttcgttggggactggcgacagacagccggctacaacctggaccaagtccttgaacagggaggtgtgtccagtttgtttcagaatctcggggtgtccgtaactccgatccaaaggattgtcctgagcggtgaaaatgggctgaagatcgacatccatgtcatcatcccgtatgaaggtctgagcggcgaccaaatgggccagatcgaaaaaatttttaaggtggtgtaccctgtggatgatcatcactttaaggtgatcctgcactatggcacactggtaatcgacggggttacgccgaacatgatcgactatttcggacggccgtatgaaggcatcgccgtgttcgacggcaaaaagatcactgtaacagggaccctgtggaacggcaacaaaattatcgacgagcgcctgatcaaccccgacggctccctgctgttccgagtaaccatcaacggagtgaccggctggcggctgtgcgaacgcattctggcgtaattctagaaaaaaaaaaaaaaaaaaaaaaaaaaaaaa

SEQ ID NO: 10 - RNA, 650 nt, synthetic construct
  misc_feature 1..650: note = NLuc mRNA
  source 1..650: mol_type = other RNA
ggcgcatattaaggtgacgcgtgtggcctcgaacaccgagcgaccctgcagcgacccgcttaaaagcttggcaatccggtactgttggtaaagccaccatggtcttcacactcgaagatttcgttggggactggcgacagacagccggctacaacctggaccaagtccttgaacagggaggtgtgtccagtttgtttcagaatctcggggtgtccgtaactccgatccaaaggattgtcctgagcggtgaaaatgggctgaagatcgacatccatgtcatcatcccgtatgaaggtctgagcggcgaccaaatgggccagatcgaaaaaatttttaaggtggtgtaccctgtggatgatcatcactttaaggtgatcctgcactatggcacactggtaatcgacggggttacgccgaacatgatcgactatttcggacggccgtatgaaggcatcgccgtgttcgacggcaaaaagatcactgtaacagggaccctgtggaacggcaacaaaattatcgacgagcgcctgatcaaccccgacggctccctgctgttccgagtaaccatcaacggagtgaccggctggcggctgtgcgaacgcattctggcgtaattctagaaaaaaaaaaaaaaaaaaaaaaaaaaaaaa

SEQ ID NO: 11 - DNA, 35 bp, synthetic construct
  misc_feature 1..35: note = DNAzyme
  source 1..35: mol_type = other DNA
ttcgaggccaggctagctacaacgaacgcgtcacc

SEQ ID NO: 12 - protein, 171 aa, synthetic construct
  REGION 1..171: note = NLuc
MVFTLEDFVGDWRQTAGYNLDQVLEQGGVSSLFQNLGVSVTPIQRIVLSGENGLKIDIHVIIPYEGLSGDQMGQIEKIFKVVYPVDDHHFKVILHYGTLVIDGVTPNMIDYFGRPYEGIAVFDGKKITVTGTLWNGNKIIDERLINPDGSLLFRVTINGVTGWRLCERILA

SEQ ID NO: 13 - DNA, 4375 bp, synthetic construct
  misc_feature 1..4375: note = Spike protein mRNA templete DNA
  source 1..4375: mol_type = other DNA
ggatgtgctgcaaggcgattaagttgggtaacgccagggttttcccagtcacgacgttgtaaaacgacggccagtgaattcgagctcggtacctcgcgaatgcatctagattaatacgactcactataggaataaactagtattcttctggtccccacagactcagagagaacccgccaccatgttcgtgttcctggtgctgctgcctctggtgtccagccagtgtgtgaacctgaccaccagaacacagctgcctccagcctacaccaacagctttaccagaggcgtgtactaccccgacaaggtgttcagatccagcgtgctgcactctacccaggacctgttcctgcctttcttcagcaacgtgacctggttccacgccatccacgtgtccggcaccaatggcaccaagagattcgacaaccccgtgctgcccttcaacgacggggtgtactttgccagcaccgagaagtccaacatcatcagaggctggatcttcggcaccacactggacagcaagacccagagcctgctgatcgtgaacaacgccaccaacgtggtcatcaaagtgtgcgagttccagttctgcaacgaccccttcctgggcgtctactaccacaagaacaacaagagctggatggaaagcgagttccgggtgtacagcagcgccaacaactgcaccttcgagtacgtgtcccagcctttcctgatggacctggaaggcaagcagggcaacttcaagaacctgcgcgagttcgtgtttaagaacatcgacggctacttcaagatctacagcaagcacacccctatcaacctcgtgcgggatctgcctcagggcttctctgctctggaacccctggtggatctgcccatcggcatcaacatcacccggtttcagacactgctggccctgcacagaagctacctgacacctggcgatagcagcagcggatggacagctggtgccgccgcttactatgtgggctacctgcagcctagaaccttcctgctgaagtacaacgagaacggcaccatcaccgacgccgtggattgtgctctggatcctctgagcgagacaaagtgcaccctgaagtccttcaccgtggaaaagggcatctaccagaccagcaacttccgggtgcagcccaccgaatccatcgtgcggttccccaatatcaccaatctgtgccccttcggcgaggtgttcaatgccaccagattcgcctctgtgtacgcctggaaccggaagcggatcagcaattgcgtggccgactactccgtgctgtacaactccgccagcttcagcaccttcaagtgctacggcgtgtcccctaccaagctgaacgacctgtgcttcacaaacgtgtacgccgacagcttcgtgatccggggagatgaagtgcggcagattgcccctggacagacaggcaagatcgccgactacaactacaagctgcccgacgacttcaccggctgtgtgattgcctggaacagcaacaacctggactccaaagtcggcggcaactacaattacctgtaccggctgttccggaagtccaatctgaagcccttcgagcgggacatctccaccgagatctatcaggccggcagcaccccttgtaacggcgtggaaggcttcaactgctacttcccactgcagtcctacggctttcagcccacaaatggcgtgggctatcagccctacagagtggtggtgctgagcttcgaactgctgcatgcccctgccacagtgtgcggccctaagaaaagcaccaatctcgtgaagaacaaatgcgtgaacttcaacttcaacggcctgaccggcaccggcgtgctgacagagagcaacaagaagttcctgccattccagcagtttggccgggatatcgccgataccacagacgccgttagagatccccagacactggaaatcctggacatcaccccttgcagcttcggcggagtgtctgtgatcacccctggcaccaacaccagcaatcaggtggcagtgctgtaccaggacgtgaactgtaccgaagtgcccgtggccattcacgccgatcagctgacacctacatggcgggtgtactccaccggcagcaatgtgtttcagaccagagccggctgtctgatcggagccgagcacgtgaacaatagctacgagtgcgacatccccatcggcgctggaatctgcgccagctaccagacacagacaaacagccctcggagagccagaagcgtggccagccagagcatcattgcctacacaatgtctctgggcgccgagaacagcgtggcctactccaacaactctatcgctatccccaccaacttcaccatcagcgtgaccacagagatcctgcctgtgtccatgaccaagaccagcgtggactgcaccatgtacatctgcggcgattccaccgagtgctccaacctgctgctgcagtacggcagcttctgcacccagctgaatagagccctgacagggatcgccgtggaacaggacaagaacacccaagaggtgttcgcccaagtgaagcagatctacaagacccctcctatcaaggacttcggcggcttcaatttcagccagattctgcccgatcctagcaagcccagcaagcggagcttcatcgaggacctgctgttcaacaaagtgacactggccgacgccggcttcatcaagcagtatggcgattgtctgggcgacattgccgccagggatctgatttgcgcccagaagtttaacggactgacagtgctgcctcctctgctgaccgatgagatgatcgcccagtacacatctgccctgctggccggcacaatcacaagcggctggacatttggagcaggcgccgctctgcagatcccctttgctatgcagatggcctaccggttcaacggcatcggagtgacccagaatgtgctgtacgagaaccagaagctgatcgccaaccagttcaacagcgccatcggcaagatccaggacagcctgagcagcacagcaagcgccctgggaaagctgcaggacgtggtcaaccagaatgcccaggcactgaacaccctggtcaagcagctgtcctccaacttcggcgccatcagctctgtgctgaacgatatcctgagcagactggaccctcctgaggccgaggtgcagatcgacagactgatcacaggcagactgcagagcctccagacatacgtgacccagcagctgatcagagccgccgagattagagcctctgccaatctggccgccaccaagatgtctgagtgtgtgctgggccagagcaagagagtggacttttgcggcaagggctaccacctgatgagcttccctcagtctgcccctcacggcgtggtgtttctgcacgtgacatatgtgcccgctcaagagaagaatttcaccaccgctccagccatctgccacgacggcaaagcccactttcctagagaaggcgtgttcgtgtccaacggcacccattggttcgtgacacagcggaacttctacgagccccagatcatcaccaccgacaacaccttcgtgtctggcaactgcgacgtcgtgatcggcattgtgaacaataccgtgtacgaccctctgcagcccgagctggacagcttcaaagaggaactggacaagtactttaagaaccacacaagccccgacgtggacctgggcgatatcagcggaatcaatgccagcgtcgtgaacatccagaaagagatcgaccggctgaacgaggtggccaagaatctgaacgagagcctgatcgacctgcaagaactggggaagtacgagcagtacatcaagtggccctggtacatctggctgggctttatcgccggactgattgccatcgtgatggtcacaatcatgctgtgttgcatgaccagctgctgtagctgcctgaagggctgttgtagctgtggcagctgctgcaagttcgacgaggacgattctgagcccgtgctgaagggcgtgaaactgcactacacatgatgactcgagctggtactgcatgcacgcaatgctagctgcccctttcccgtcctgggtaccccgagtctcccccgacctcgggtcccaggtatgctcccacctccacctgccccactcaccacctctgctagttccagacacctcccaagcacgcagcaatgcagctcaaaacgcttagcctagccacacccccacgggaaacagcagtgattaacctttagcaataaacgaaagtttaactaagctatactaaccccagggttggtcaatttcgtgccagccacaccctggaaaaaaaaaaaaaaaaaaaaaaaaaaaaaaaaaaaaaaaaaaaaaaaaaaaaaaaaaaaaaaaaaaaaaaaaaaaaaaaaa

SEQ ID NO: 14 - RNA, 4247 nt, synthetic construct
  misc_feature 1..4247: note = Spike protein mRNA
  source 1..4247: mol_type = other RNA
ggaataaactagtattcttctggtccccacagactcagagagaacccgccaccatgttcgtgttcctggtgctgctgcctctggtgtccagccagtgtgtgaacctgaccaccagaacacagctgcctccagcctacaccaacagctttaccagaggcgtgtactaccccgacaaggtgttcagatccagcgtgctgcactctacccaggacctgttcctgcctttcttcagcaacgtgacctggttccacgccatccacgtgtccggcaccaatggcaccaagagattcgacaaccccgtgctgcccttcaacgacggggtgtactttgccagcaccgagaagtccaacatcatcagaggctggatcttcggcaccacactggacagcaagacccagagcctgctgatcgtgaacaacgccaccaacgtggtcatcaaagtgtgcgagttccagttctgcaacgaccccttcctgggcgtctactaccacaagaacaacaagagctggatggaaagcgagttccgggtgtacagcagcgccaacaactgcaccttcgagtacgtgtcccagcctttcctgatggacctggaaggcaagcagggcaacttcaagaacctgcgcgagttcgtgtttaagaacatcgacggctacttcaagatctacagcaagcacacccctatcaacctcgtgcgggatctgcctcagggcttctctgctctggaacccctggtggatctgcccatcggcatcaacatcacccggtttcagacactgctggccctgcacagaagctacctgacacctggcgatagcagcagcggatggacagctggtgccgccgcttactatgtgggctacctgcagcctagaaccttcctgctgaagtacaacgagaacggcaccatcaccgacgccgtggattgtgctctggatcctctgagcgagacaaagtgcaccctgaagtccttcaccgtggaaaagggcatctaccagaccagcaacttccgggtgcagcccaccgaatccatcgtgcggttccccaatatcaccaatctgtgccccttcggcgaggtgttcaatgccaccagattcgcctctgtgtacgcctggaaccggaagcggatcagcaattgcgtggccgactactccgtgctgtacaactccgccagcttcagcaccttcaagtgctacggcgtgtcccctaccaagctgaacgacctgtgcttcacaaacgtgtacgccgacagcttcgtgatccggggagatgaagtgcggcagattgcccctggacagacaggcaagatcgccgactacaactacaagctgcccgacgacttcaccggctgtgtgattgcctggaacagcaacaacctggactccaaagtcggcggcaactacaattacctgtaccggctgttccggaagtccaatctgaagcccttcgagcgggacatctccaccgagatctatcaggccggcagcaccccttgtaacggcgtggaaggcttcaactgctacttcccactgcagtcctacggctttcagcccacaaatggcgtgggctatcagccctacagagtggtggtgctgagcttcgaactgctgcatgcccctgccacagtgtgcggccctaagaaaagcaccaatctcgtgaagaacaaatgcgtgaacttcaacttcaacggcctgaccggcaccggcgtgctgacagagagcaacaagaagttcctgccattccagcagtttggccgggatatcgccgataccacagacgccgttagagatccccagacactggaaatcctggacatcaccccttgcagcttcggcggagtgtctgtgatcacccctggcaccaacaccagcaatcaggtggcagtgctgtaccaggacgtgaactgtaccgaagtgcccgtggccattcacgccgatcagctgacacctacatggcgggtgtactccaccggcagcaatgtgtttcagaccagagccggctgtctgatcggagccgagcacgtgaacaatagctacgagtgcgacatccccatcggcgctggaatctgcgccagctaccagacacagacaaacagccctcggagagccagaagcgtggccagccagagcatcattgcctacacaatgtctctgggcgccgagaacagcgtggcctactccaacaactctatcgctatccccaccaacttcaccatcagcgtgaccacagagatcctgcctgtgtccatgaccaagaccagcgtggactgcaccatgtacatctgcggcgattccaccgagtgctccaacctgctgctgcagtacggcagcttctgcacccagctgaatagagccctgacagggatcgccgtggaacaggacaagaacacccaagaggtgttcgcccaagtgaagcagatctacaagacccctcctatcaaggacttcggcggcttcaatttcagccagattctgcccgatcctagcaagcccagcaagcggagcttcatcgaggacctgctgttcaacaaagtgacactggccgacgccggcttcatcaagcagtatggcgattgtctgggcgacattgccgccagggatctgatttgcgcccagaagtttaacggactgacagtgctgcctcctctgctgaccgatgagatgatcgcccagtacacatctgccctgctggccggcacaatcacaagcggctggacatttggagcaggcgccgctctgcagatcccctttgctatgcagatggcctaccggttcaacggcatcggagtgacccagaatgtgctgtacgagaaccagaagctgatcgccaaccagttcaacagcgccatcggcaagatccaggacagcctgagcagcacagcaagcgccctgggaaagctgcaggacgtggtcaaccagaatgcccaggcactgaacaccctggtcaagcagctgtcctccaacttcggcgccatcagctctgtgctgaacgatatcctgagcagactggaccctcctgaggccgaggtgcagatcgacagactgatcacaggcagactgcagagcctccagacatacgtgacccagcagctgatcagagccgccgagattagagcctctgccaatctggccgccaccaagatgtctgagtgtgtgctgggccagagcaagagagtggacttttgcggcaagggctaccacctgatgagcttccctcagtctgcccctcacggcgtggtgtttctgcacgtgacatatgtgcccgctcaagagaagaatttcaccaccgctccagccatctgccacgacggcaaagcccactttcctagagaaggcgtgttcgtgtccaacggcacccattggttcgtgacacagcggaacttctacgagccccagatcatcaccaccgacaacaccttcgtgtctggcaactgcgacgtcgtgatcggcattgtgaacaataccgtgtacgaccctctgcagcccgagctggacagcttcaaagaggaactggacaagtactttaagaaccacacaagccccgacgtggacctgggcgatatcagcggaatcaatgccagcgtcgtgaacatccagaaagagatcgaccggctgaacgaggtggccaagaatctgaacgagagcctgatcgacctgcaagaactggggaagtacgagcagtacatcaagtggccctggtacatctggctgggctttatcgccggactgattgccatcgtgatggtcacaatcatgctgtgttgcatgaccagctgctgtagctgcctgaagggctgttgtagctgtggcagctgctgcaagttcgacgaggacgattctgagcccgtgctgaagggcgtgaaactgcactacacatgatgactcgagctggtactgcatgcacgcaatgctagctgcccctttcccgtcctgggtaccccgagtctcccccgacctcgggtcccaggtatgctcccacctccacctgccccactcaccacctctgctagttccagacacctcccaagcacgcagcaatgcagctcaaaacgcttagcctagccacacccccacgggaaacagcagtgattaacctttagcaataaacgaaagtttaactaagctatactaaccccagggttggtcaatttcgtgccagccacaccctggaaaaaaaaaaaaaaaaaaaaaaaaaaaaaaaaaaaaaaaaaaaaaaaaaaaaaaaaaaaaaaaaaaaaaaaaaaaaaaaaa

SEQ ID NO: 15 - RNA, 19 nt, synthetic construct
  misc_feature 1..19: note = artificial sequence
  source 1..19: mol_type = other RNA
gaacgtgcgaaagtccaca

SEQ ID NO: 16 - RNA, 106 nt, synthetic construct
  misc_feature 1..106: note = artificial sequence
  misc_feature 1: note = The 5' end is modified with a cap, which is protected by aphotodegradable protecting group.
  source 1..106: mol_type = other RNA
gagccaccatggactacaaggacgacgacgataagatcatcgactataaagacgacgacgataaacaccaccaccaccaccactgaaaaaaaaaaaaaaaaaaaaa

SEQ ID NO: 17 - RNA, 130 nt, synthetic construct
  misc_feature 1..130: note = artificial sequence
  misc_feature 1: note = The 5' end is modified with a cap, which is protected by aphotodegradable protecting group.
  source 1..130: mol_type = other RNA
gagccaccatgggatggagctgtatcatcctcttcttggtagcaacagctacaggcgcgcactccagtataatcaactttgaaaaactgagcgagaaggacgagctgtagaaaaaaaaaaaaaaaaaaaa

SEQ ID NO: 18 - DNA, 28 bp, synthetic construct
  misc_feature 1..28: note = T7 promoter
  source 1..28: mol_type = other DNA
cccggatcctaatacgactcactatagg

SEQ ID NO: 19 - DNA, 39 bp, synthetic construct
  misc_feature 1..39: note = DNAzyme
  source 1..39: mol_type = other DNA
tctgtggggaggctagctacaacgacagaagaatactag